European Patent Application EP 4 477 739 A1, published December 18, 2024. Title: セルロース合成微生物の形質転換体およびその使用. Applicant: SUMITOMO CHEMICAL COMPANY, LIMITED. The sequence listing filed with the application follows.

SEQUENCE LISTING (27 sequences)

SEQ ID NO: 1 - DNA, 228 bp, synthetic construct
  misc_feature 1..228: note = oprI
  source 1..228: mol_type = other DNA
atgaacaacgttctgaaattctctgctctggctctggctgctgttctggccaccggttgcagcagccactccaaagaaaccgaagctcgtctgaccgctaccgaagacgcagctgctcgtgctcaggctcgcgctgacgaagcctatcgcaaggctgacgaagctctgggcgctgctcagaaagctcagcagactgctgacgaggctaacgagcgtgccctgcgcatg

SEQ ID NO: 2 - protein, 76 aa, synthetic construct
  REGION 1..76: note = amino acid of oprI
MNNVLKFSALALAAVLATGCSSHSKETEARLTATEDAAARAQARADEAYRKADEALGAAQKAQQTADEANERALRM

SEQ ID NO: 3 - DNA, 717 bp, synthetic construct
  misc_feature 1..717: note = GFP
  source 1..717: mol_type = other DNA
atgagtaaaggagaagaacttttcactggagttgtcccaattcttgttgaattagatggtgatgttaatgggcacaaattttctgtcagtggagagggtgaaggtgatgcaacatacggaaaacttacccttaaatttatttgcactactggaaaactacctgttccatggccaacacttgtcactactttgacttatggtgttcaatgcttttcaagatacccagatcatatgaaacggcatgactttttcaagagtgccatgcccgaaggttatgtacaggaaagaactatatttttcaaagatgacgggaactataagacacgtgctgaagtcaagtttgaaggtgatacacttgttaatagaatcgagttaaaaggtattgattttaaagaagatggaaacattcttggacacaaattggaatacaactataactcacacaatgtatacatcatggcagacaaacaaaagaatggaatcaaagttaacttcaaaattagacacaacattgaagatggaagcgttcaactagcagaccattatcaacaaaatactccaattggcgatggccctgtccttttaccagacaaccattacctgtccacacaatctgccctttcgaaagatcccaacgaaaagagagaccacatggtccttcttgagtttgtaacagctgctgggattacacatggcatggatgaactatacaaatga

SEQ ID NO: 4 - DNA, 1452 bp, synthetic construct
  misc_feature 1..1452: note = bglC
  source 1..1452: mol_type = other DNA
atgaccagccaaagtaccaccccgctgggtaacctggaagaaaccccgaaacctgacatccgtttcccgagtgattttgtgtggggcgtggcaaccgcaagcttccagatcgaaggtagtaccaccgcagatggtcgcggtccgagtatttgggatacattctgtgccaccccgggtaaagttgagaacggcgataccggtgacccggcatgcgatcattacaaccgctatcgcgatgatgtggcactgatgcgtgaactgggcgttggtgcctatcgctttagcatcgcatggccgcgtattcagcctgagggtaagggtaccccggttgaagccggcctggatttttatgaccgcctggtggactgtctgctggaagccggcatcgagccgtggccgacactgtatcattgggatctgccgcaggcactggaagatgccggtggttggccgaatcgcgatacagccaagcgctttgccgattatgccgagatcgtgtaccgtcgtctgggcgatcgcatcacaaactggaacaccctgaacgaaccttggtgtagtgcctttctgggctatgcaagcggtgttcatgccccgggtcgtcaagaaccggccgcagcactggcagcagcacatcacctgatgttaggtcatggtctggcagccgcagttatgcgcgatttagcaggccaggcaggtcgcagcgttcgcattggcgtggcacataaccagaccaccgttcgcccgtataccgatagtgaagccgatcgcgatgcagcccgtcgtattgacgcactgcgcaaccgcattttcaccgaaccgctggtgaaaggccgctatccggaggacttaattgaggacgtggcagccgtgaccgactatagctttgtgcaggacggcgatctgaagaccatcagcgccaatctggacatgatgggtgtgaacttttacaacccgagctgggttagcggcaatcgcgagaatggcggtagtgatcgtctgccggatgaaggctatagtccgagcgtgggcagtgagcacgtggtggaagttgacccgggtctgcctgtgaccgcaatgggttggccgattgatccgacaggcctgtatgatacactgacacgcctggccaatgactatcctggcctgcctctgtacatcaccgagaacggcgcagcctttgaggataaagtggttgacggcgccgtgcatgataccgagcgcattgcctatctggatagccatctgcgcgcagcacacgcagccattgaggccggtgttccgctgaaaggttatttcgcctggagcttcatggacaacttcgagtgggcactgggttatggcaaacgcttcggtatcgtgcatgttgattacgagagccagacccgcaccgtgaaagatagtggctggtggtacagccgtgttatgcgtaacggtggcatttttggccaggaa

SEQ ID NO: 5 - DNA, 1335 bp, synthetic construct
  misc_feature 1..1335: note = cex
  source 1..1335: mol_type = other DNA
atgcctaggaccacgcccgcacccggccacccggcccgcggcgcccgcaccgctctgcgcacgacgctcgccgccgcggcggcgacgctcgtcgtcggcgccacggtcgtgctgcccgcccaggccgcgaccacgctcaaggaggccgccgacggcgccggccgggacttcggcttcgcgctcgaccccaaccggctctcggaggcgcagtacaaggcgatcgccgacagcgagttcaacctcgtcgtcgccgagaacgcgatgaagtgggacgccaccgagccctcgcagaacagcttctccttcggcgcgggcgaccgcgtcgcgagctacgccgccgacaccggcaaggagctgtacggccacacgctcgtctggcactcgcagctgcccgactgggcgaagaacctcaacggctccgcgttcgagagcgcgatggtcaaccacgtgacgaaggtcgccgaccacttcgagggcaaggtcgcgtcgtgggacgtcgtcaacgaggcgttcgccgacggcggcggccgccggcaggactcggcgttccagcagaagctcggcaacggctacatcgagaccgcgttccgggcggcacgtgcggcggacccgaccgccaagctgtgcatcaacgactacaacgtcgagggcatcaacgcgaagagcaactcgctctacgacctcgtcaaggacttcaaggcgcgcggcgtcccgctcgactgcgtcgggttccagtcgcacctcatcgtcggccaggtgccgggcgacttccggcagaacctgcagcggttcgcggacctgggcgtggacgtgcgcatcaccgagctcgacatccgcatgcggacgccctccgacgcgaccaagctcgcgacccaggcggccgactacaagaaggtcgtgcaggcctgcatgcaggtgacccgctgccagggcgtgaccgtctggggcatcaccgacaagtactcgtgggtgccggacgtcttcccgggcgagggggccgcgctggtgtgggacgcgagctacgccaagaagccggcctacgccgccgtgatggaggccttcggcgcgagcccgacgccgacgcccaccacgccgaccccgacgcccacgacgccgacgccgaccccgacgtccggtccggccgggtgccaggtgctgtggggcgtcaaccagtggaacaccggcttcaccgcgaacgtcaccgtgaagaacacgtcctccgctccggtcgacggctggacgctcacgttcagcttcccgtccggccagcaggtcacccaggcgtggagctcgacggtcacgcagtccggctcggccgtgacggtccgcaacgcc

SEQ ID NO: 6 - DNA, 1053 bp, synthetic construct
  misc_feature 1..1053: note = cenA
  source 1..1053: mol_type = other DNA
aacggcagcatcccgaccggcggcacggcgtcgttcgggttcaacggctcgtgggccgggtccaacccgacgccggcgtcgttctcgctcaacggcaccacctgcacgggcaccgtgccgacgaccagccccacgccgaccccgacgccgacgacccccacgccgacgccgaccccgacccccacccccacgccgacggtcacgccgcagccgaccagcggcttctacgtcgacccgacgacgcagggctaccgcgcgtggcaggccgcgtccggcacggacaaggcgctgctcgagaagatcgcgctcaccccgcaggcgtactgggtcggcaactgggccgacgcgtcgcacgcgcaggccgaggtcgccgactacaccggccgcgccgtcgcggccgggaagacgccgatgctcgtcgtctacgcgatcccgggccgcgactgcggctcgcactccggcggtggtgtgtccgagtccgagtacgcgcgctgggtcgacaccgtcgcgcagggcatcaagggcaacccgatcgtgatcctcgagcccgacgcgctcgcgcagctcggcgactgctccggccagggtgaccgcgtcggcttcctcaagtacgccgccaagtcgctcaccctcaagggcgcgcgcgtctacatcgacgcgggccacgcgaagtggctgtcggtcgacaccgcggtgaaccgcctcaaccaggtcggcttcgagtacgcggtgggcttcgcgctcaacacgtcgaactaccagacgacggcggacagcaaggcgtacggccagcagatctcgcagcggctgggcggcaagaagttcgtcatcgacacctcgcgcaacggcaacggctcgaacggcgagtggtgcaacccgcgcggccgcgcgctcggcgaacgcccggtcgcggtgaacgacggctccggcctggacgcgctcctgtgggtcaagctgcccggcgagtccgacggcgcgtgcaacggcggcccggccgccggccagtggtggcaggagatcgccctggagatggcgcgcaacgccaggtggtga

SEQ ID NO: 7 - DNA, 945 bp, synthetic construct
  misc_feature 1..945: note = oprI-gfp
  source 1..945: mol_type = other DNA
atgaacaacgttctgaaattctctgctctggctctggctgctgttctggccaccggttgcagcagccactccaaagaaaccgaagctcgtctgaccgctaccgaagacgcagctgctcgtgctcaggctcgcgctgacgaagcctatcgcaaggctgacgaagctctgggcgctgctcagaaagctcagcagactgctgacgaggctaacgagcgtgccctgcgcatgatgagtaaaggagaagaacttttcactggagttgtcccaattcttgttgaattagatggtgatgttaatgggcacaaattttctgtcagtggagagggtgaaggtgatgcaacatacggaaaacttacccttaaatttatttgcactactggaaaactacctgttccatggccaacacttgtcactactttgacttatggtgttcaatgcttttcaagatacccagatcatatgaaacggcatgactttttcaagagtgccatgcccgaaggttatgtacaggaaagaactatatttttcaaagatgacgggaactataagacacgtgctgaagtcaagtttgaaggtgatacacttgttaatagaatcgagttaaaaggtattgattttaaagaagatggaaacattcttggacacaaattggaatacaactataactcacacaatgtatacatcatggcagacaaacaaaagaatggaatcaaagttaacttcaaaattagacacaacattgaagatggaagcgttcaactagcagaccattatcaacaaaatactccaattggcgatggccctgtccttttaccagacaaccattacctgtccacacaatctgccctttcgaaagatcccaacgaaaagagagaccacatggtccttcttgagtttgtaacagctgctgggattacacatggcatggatgaactatacaaatga

SEQ ID NO: 8 - DNA, 4119 bp, synthetic construct
  misc_feature 1..4119: note = oprI-bglC-cex-cenA
  source 1..4119: mol_type = other DNA
atgaacaacgttctgaaattctctgctctggctctggctgctgttctggccaccggttgcagcagccactccaaagaaaccgaagctcgtctgaccgctaccgaagacgcagctgctcgtgctcaggctcgcgctgacgaagcctatcgcaaggctgacgaagctctgggcgctgctcagaaagctcagcagactgctgacgaggctaacgagcgtgccctgcgcatgatgaccagccaaagtaccaccccgctgggtaacctggaagaaaccccgaaacctgacatccgtttcccgagtgattttgtgtggggcgtggcaaccgcaagcttccagatcgaaggtagtaccaccgcagatggtcgcggtccgagtatttgggatacattctgtgccaccccgggtaaagttgagaacggcgataccggtgacccggcatgcgatcattacaaccgctatcgcgatgatgtggcactgatgcgtgaactgggcgttggtgcctatcgctttagcatcgcatggccgcgtattcagcctgagggtaagggtaccccggttgaagccggcctggatttttatgaccgcctggtggactgtctgctggaagccggcatcgagccgtggccgacactgtatcattgggatctgccgcaggcactggaagatgccggtggttggccgaatcgcgatacagccaagcgctttgccgattatgccgagatcgtgtaccgtcgtctgggcgatcgcatcacaaactggaacaccctgaacgaaccttggtgtagtgcctttctgggctatgcaagcggtgttcatgccccgggtcgtcaagaaccggccgcagcactggcagcagcacatcacctgatgttaggtcatggtctggcagccgcagttatgcgcgatttagcaggccaggcaggtcgcagcgttcgcattggcgtggcacataaccagaccaccgttcgcccgtataccgatagtgaagccgatcgcgatgcagcccgtcgtattgacgcactgcgcaaccgcattttcaccgaaccgctggtgaaaggccgctatccggaggacttaattgaggacgtggcagccgtgaccgactatagctttgtgcaggacggcgatctgaagaccatcagcgccaatctggacatgatgggtgtgaacttttacaacccgagctgggttagcggcaatcgcgagaatggcggtagtgatcgtctgccggatgaaggctatagtccgagcgtgggcagtgagcacgtggtggaagttgacccgggtctgcctgtgaccgcaatgggttggccgattgatccgacaggcctgtatgatacactgacacgcctggccaatgactatcctggcctgcctctgtacatcaccgagaacggcgcagcctttgaggataaagtggttgacggcgccgtgcatgataccgagcgcattgcctatctggatagccatctgcgcgcagcacacgcagccattgaggccggtgttccgctgaaaggttatttcgcctggagcttcatggacaacttcgagtgggcactgggttatggcaaacgcttcggtatcgtgcatgttgattacgagagccagacccgcaccgtgaaagatagtggctggtggtacagccgtgttatgcgtaacggtggcatttttggccaggaaggtggcggtggctcgggcggtggtgggtcgggtggcggtggctcgatgcctaggaccacgcccgcacccggccacccggcccgcggcgcccgcaccgctctgcgcacgacgctcgccgccgcggcggcgacgctcgtcgtcggcgccacggtcgtgctgcccgcccaggccgcgaccacgctcaaggaggccgccgacggcgccggccgggacttcggcttcgcgctcgaccccaaccggctctcggaggcgcagtacaaggcgatcgccgacagcgagttcaacctcgtcgtcgccgagaacgcgatgaagtgggacgccaccgagccctcgcagaacagcttctccttcggcgcgggcgaccgcgtcgcgagctacgccgccgacaccggcaaggagctgtacggccacacgctcgtctggcactcgcagctgcccgactgggcgaagaacctcaacggctccgcgttcgagagcgcgatggtcaaccacgtgacgaaggtcgccgaccacttcgagggcaaggtcgcgtcgtgggacgtcgtcaacgaggcgttcgccgacggcggcggccgccggcaggactcggcgttccagcagaagctcggcaacggctacatcgagaccgcgttccgggcggcacgtgcggcggacccgaccgccaagctgtgcatcaacgactacaacgtcgagggcatcaacgcgaagagcaactcgctctacgacctcgtcaaggacttcaaggcgcgcggcgtcccgctcgactgcgtcgggttccagtcgcacctcatcgtcggccaggtgccgggcgacttccggcagaacctgcagcggttcgcggacctgggcgtggacgtgcgcatcaccgagctcgacatccgcatgcggacgccctccgacgcgaccaagctcgcgacccaggcggccgactacaagaaggtcgtgcaggcctgcatgcaggtgacccgctgccagggcgtgaccgtctggggcatcaccgacaagtactcgtgggtgccggacgtcttcccgggcgagggggccgcgctggtgtgggacgcgagctacgccaagaagccggcctacgccgccgtgatggaggccttcggcgcgagcccgacgccgacgcccaccacgccgaccccgacgcccacgacgccgacgccgaccccgacgtccggtccggccgggtgccaggtgctgtggggcgtcaaccagtggaacaccggcttcaccgcgaacgtcaccgtgaagaacacgtcctccgctccggtcgacggctggacgctcacgttcagcttcccgtccggccagcaggtcacccaggcgtggagctcgacggtcacgcagtccggctcggccgtgacggtccgcaacgccccatggaacggcagcatcccgaccggcggcacggcgtcgttcgggttcaacggctcgtgggccgggtccaacccgacgccggcgtcgttctcgctcaacggcaccacctgcacgggcaccgtgccgacgaccagccccacgccgaccccgacgccgacgacccccacgccgacgccgaccccgacccccacccccacgccgacggtcacgccgcagccgaccagcggcttctacgtcgacccgacgacgcagggctaccgcgcgtggcaggccgcgtccggcacggacaaggcgctgctcgagaagatcgcgctcaccccgcaggcgtactgggtcggcaactgggccgacgcgtcgcacgcgcaggccgaggtcgccgactacaccggccgcgccgtcgcggccgggaagacgccgatgctcgtcgtctacgcgatcccgggccgcgactgcggctcgcactccggcggtggtgtgtccgagtccgagtacgcgcgctgggtcgacaccgtcgcgcagggcatcaagggcaacccgatcgtgatcctcgagcccgacgcgctcgcgcagctcggcgactgctccggccagggtgaccgcgtcggcttcctcaagtacgccgccaagtcgctcaccctcaagggcgcgcgcgtctacatcgacgcgggccacgcgaagtggctgtcggtcgacaccgcggtgaaccgcctcaaccaggtcggcttcgagtacgcggtgggcttcgcgctcaacacgtcgaactaccagacgacggcggacagcaaggcgtacggccagcagatctcgcagcggctgggcggcaagaagttcgtcatcgacacctcgcgcaacggcaacggctcgaacggcgagtggtgcaacccgcgcggccgcgcgctcggcgaacgcccggtcgcggtgaacgacggctccggcctggacgcgctcctgtgggtcaagctgcccggcgagtccgacggcgcgtgcaacggcggcccggccgccggccagtggtggcaggagatcgccctggagatggcgcgcaacgccaggtggtga

SEQ ID NO: 9 - DNA, 2622 bp, synthetic construct
  misc_feature 1..2622: note = oprI-cex-cenA
  source 1..2622: mol_type = other DNA
atgaacaacgttctgaaattctctgctctggctctggctgctgttctggccaccggttgcagcagccactccaaagaaaccgaagctcgtctgaccgctaccgaagacgcagctgctcgtgctcaggctcgcgctgacgaagcctatcgcaaggctgacgaagctctgggcgctgctcagaaagctcagcagactgctgacgaggctaacgagcgtgccctgcgcatgatgcctaggaccacgcccgcacccggccacccggcccgcggcgcccgcaccgctctgcgcacgacgctcgccgccgcggcggcgacgctcgtcgtcggcgccacggtcgtgctgcccgcccaggccgcgaccacgctcaaggaggccgccgacggcgccggccgggacttcggcttcgcgctcgaccccaaccggctctcggaggcgcagtacaaggcgatcgccgacagcgagttcaacctcgtcgtcgccgagaacgcgatgaagtgggacgccaccgagccctcgcagaacagcttctccttcggcgcgggcgaccgcgtcgcgagctacgccgccgacaccggcaaggagctgtacggccacacgctcgtctggcactcgcagctgcccgactgggcgaagaacctcaacggctccgcgttcgagagcgcgatggtcaaccacgtgacgaaggtcgccgaccacttcgagggcaaggtcgcgtcgtgggacgtcgtcaacgaggcgttcgccgacggcggcggccgccggcaggactcggcgttccagcagaagctcggcaacggctacatcgagaccgcgttccgggcggcacgtgcggcggacccgaccgccaagctgtgcatcaacgactacaacgtcgagggcatcaacgcgaagagcaactcgctctacgacctcgtcaaggacttcaaggcgcgcggcgtcccgctcgactgcgtcgggttccagtcgcacctcatcgtcggccaggtgccgggcgacttccggcagaacctgcagcggttcgcggacctgggcgtggacgtgcgcatcaccgagctcgacatccgcatgcggacgccctccgacgcgaccaagctcgcgacccaggcggccgactacaagaaggtcgtgcaggcctgcatgcaggtgacccgctgccagggcgtgaccgtctggggcatcaccgacaagtactcgtgggtgccggacgtcttcccgggcgagggggccgcgctggtgtgggacgcgagctacgccaagaagccggcctacgccgccgtgatggaggccttcggcgcgagcccgacgccgacgcccaccacgccgaccccgacgcccacgacgccgacgccgaccccgacgtccggtccggccgggtgccaggtgctgtggggcgtcaaccagtggaacaccggcttcaccgcgaacgtcaccgtgaagaacacgtcctccgctccggtcgacggctggacgctcacgttcagcttcccgtccggccagcaggtcacccaggcgtggagctcgacggtcacgcagtccggctcggccgtgacggtccgcaacgccccatggaacggcagcatcccgaccggcggcacggcgtcgttcgggttcaacggctcgtgggccgggtccaacccgacgccggcgtcgttctcgctcaacggcaccacctgcacgggcaccgtgccgacgaccagccccacgccgaccccgacgccgacgacccccacgccgacgccgaccccgacccccacccccacgccgacggtcacgccgcagccgaccagcggcttctacgtcgacccgacgacgcagggctaccgcgcgtggcaggccgcgtccggcacggacaaggcgctgctcgagaagatcgcgctcaccccgcaggcgtactgggtcggcaactgggccgacgcgtcgcacgcgcaggccgaggtcgccgactacaccggccgcgccgtcgcggccgggaagacgccgatgctcgtcgtctacgcgatcccgggccgcgactgcggctcgcactccggcggtggtgtgtccgagtccgagtacgcgcgctgggtcgacaccgtcgcgcagggcatcaagggcaacccgatcgtgatcctcgagcccgacgcgctcgcgcagctcggcgactgctccggccagggtgaccgcgtcggcttcctcaagtacgccgccaagtcgctcaccctcaagggcgcgcgcgtctacatcgacgcgggccacgcgaagtggctgtcggtcgacaccgcggtgaaccgcctcaaccaggtcggcttcgagtacgcggtgggcttcgcgctcaacacgtcgaactaccagacgacggcggacagcaaggcgtacggccagcagatctcgcagcggctgggcggcaagaagttcgtcatcgacacctcgcgcaacggcaacggctcgaacggcgagtggtgcaacccgcgcggccgcgcgctcggcgaacgcccggtcgcggtgaacgacggctccggcctggacgcgctcctgtgggtcaagctgcccggcgagtccgacggcgcgtgcaacggcggcccggccgccggccagtggtggcaggagatcgccctggagatggcgcgcaacgccaggtggtga

SEQ ID NO: 10 - protein, 484 aa, synthetic construct
  REGION 1..484: note = Beta-glucosidase
MTSQSTTPLGNLEETPKPDIRFPSDFVWGVATASFQIEGSTTADGRGPSIWDTFCATPGKVENGDTGDPACDHYNRYRDDVALMRELGVGAYRFSIAWPRIQPEGKGTPVEAGLDFYDRLVDCLLEAGIEPWPTLYHWDLPQALEDAGGWPNRDTAKRFADYAEIVYRRLGDRITNWNTLNEPWCSAFLGYASGVHAPGRQEPAAALAAAHHLMLGHGLAAAVMRDLAGQAGRSVRIGVAHNQTTVRPYTDSEADRDAARRIDALRNRIFTEPLVKGRYPEDLIEDVAAVTDYSFVQDGDLKTISANLDMMGVNFYNPSWVSGNRENGGSDRLPDEGYSPSVGSEHVVEVDPGLPVTAMGWPIDPTGLYDTLTRLANDYPGLPLYITENGAAFEDKVVDGAVHDTERIAYLDSHLRAAHAAIEAGVPLKGYFAWSFMDNFEWALGYGKRFGIVHVDYESQTRTVKDSGWWYSRVMRNGGIFGQE

SEQ ID NO: 11 - protein, 445 aa, synthetic construct
  REGION 1..445: note = Exoglucanase
MPRTTPAPGHPARGARTALRTTLAAAAATLVVGATVVLPAQAATTLKEAADGAGRDFGFALDPNRLSEAQYKAIADSEFNLVVAENAMKWDATEPSQNSFSFGAGDRVASYAADTGKELYGHTLVWHSQLPDWAKNLNGSAFESAMVNHVTKVADHFEGKVASWDVVNEAFADGGGRRQDSAFQQKLGNGYIETAFRAARAADPTAKLCINDYNVEGINAKSNSLYDLVKDFKARGVPLDCVGFQSHLIVGQVPGDFRQNLQRFADLGVDVRITELDIRMRTPSDATKLATQAADYKKVVQACMQVTRCQGVTVWGITDKYSWVPDVFPGEGAALVWDASYAKKPAYAAVMEAFGASPTPTPTTPTPTPTTPTPTPTSGPAGCQVLWGVNQWNTGFTANVTVKNTSSAPVDGWTLTFSFPSGQQVTQAWSSTVTQSGSAVTVRNA

SEQ ID NO: 12 - protein, 350 aa, synthetic construct
  REGION 1..350: note = Endoglucanase
NGSIPTGGTASFGFNGSWAGSNPTPASFSLNGTTCTGTVPTTSPTPTPTPTTPTPTPTPTPTPTPTVTPQPTSGFYVDPTTQGYRAWQAASGTDKALLEKIALTPQAYWVGNWADASHAQAEVADYTGRAVAAGKTPMLVVYAIPGRDCGSHSGGGVSESEYARWVDTVAQGIKGNPIVILEPDALAQLGDCSGQGDRVGFLKYAAKSLTLKGARVYIDAGHAKWLSVDTAVNRLNQVGFEYAVGFALNTSNYQTTADSKAYGQQISQRLGGKKFVIDTSRNGNGSNGEWCNPRGRALGERPVAVNDGSGLDALLWVKLPGESDGACNGGPAAGQWWQEIALEMARNARW

SEQ ID NO: 13 - DNA, 29 bp, synthetic construct
  misc_feature 1..29: note = pTE105-KpnI-F1
  source 1..29: mol_type = other DNA
ggtacctaattcactggccgtcgttttac

SEQ ID NO: 14 - DNA, 33 bp, synthetic construct
  misc_feature 1..33: note = pTE105-SpeI-R1
  source 1..33: mol_type = other DNA
actagtcaagatctaagcttcgtgcaatcctac

SEQ ID NO: 15 - DNA, 54 bp, synthetic construct
  misc_feature 1..54: note = gfp-SpeI-RBS-F1
  source 1..54: mol_type = other DNA
aagcttagatcttgactagtaaggagatcgagcatatgagtaaaggagaagaac

SEQ ID NO: 16 - DNA, 43 bp, synthetic construct
  misc_feature 1..43: note = gfp-KpnI-R1
  source 1..43: mol_type = other DNA
cggccagtgaattaggtaccctatttgtatagttcatccatgc

SEQ ID NO: 17 - DNA, 66 bp, synthetic construct
  misc_feature 1..66: note = oprI-SpeI-RBS-F1
  source 1..66: mol_type = other DNA
aagcttagatcttgactagtaaggagatcgagcatatgaacaacgttctgaaattctctgctctgg

SEQ ID NO: 18 - DNA, 28 bp, synthetic construct
  misc_feature 1..28: note = oprI-R1
  source 1..28: mol_type = other DNA
ctttactcatcatgcgcagggcacgctc

SEQ ID NO: 19 - DNA, 29 bp, synthetic construct
  misc_feature 1..29: note = gfp-F2
  source 1..29: mol_type = other DNA
cctgcgcatgatgagtaaaggagaagaac

SEQ ID NO: 20 - DNA, 38 bp, synthetic construct
  misc_feature 1..38: note = bglC-F1
  source 1..38: mol_type = other DNA
acgagcgtgccctgcgcatgatgaccagccaaagtacc

SEQ ID NO: 21 - DNA, 83 bp, synthetic construct
  misc_feature 1..83: note = bglC-R1
  source 1..83: mol_type = other DNA
gcgggcgtggtcctaggcatcgagccaccgccacccgacccaccaccgcccgagccaccgccaccttcctggccaaaaatgcc

SEQ ID NO: 22 - DNA, 18 bp, synthetic construct
  misc_feature 1..18: note = cex-F1
  source 1..18: mol_type = other DNA
atgcctaggaccacgccc

SEQ ID NO: 23 - DNA, 28 bp, synthetic construct
  misc_feature 1..28: note = cex-R1
  source 1..28: mol_type = other DNA
cgttccatggggcgttgcggaccgtcac

SEQ ID NO: 24 - DNA, 34 bp, synthetic construct
  misc_feature 1..34: note = cenA-F1
  source 1..34: mol_type = other DNA
ccgcaacgccccatggaacggcagcatcccgacc

SEQ ID NO: 25 - DNA, 38 bp, synthetic construct
  misc_feature 1..38: note = cenA-R1
  source 1..38: mol_type = other DNA
cggccagtgaattaggtacctcaccacctggcgttgcg

SEQ ID NO: 26 - DNA, 18 bp, synthetic construct
  misc_feature 1..18: note = oprI-R2
  source 1..18: mol_type = other DNA
catgcgcagggcacgctc

SEQ ID NO: 27 - DNA, 33 bp, synthetic construct
  misc_feature 1..33: note = cex-F2
  source 1..33: mol_type = other DNA
cgtgccctgcgcatgatgcctaggaccacgccc